European Patent Application EP 4 495 245 A1, published January 22, 2025. Title: MHC gene-humanized animals. Applicant: Tokyo Metropolitan Institute of Medical Science. The sequence listing filed with the application follows.

SEQUENCE LISTING (52 sequences)

SEQ ID NO: 1 - DNA, 5327 bp, synthetic construct
  misc_feature 1..5327: note = Synthetic DNA
  misc_feature 30..1217: note = /label="EF1"
  misc_feature 1230..2267: note = /label="Hyg"
  misc_feature 2274..2808: note = /label="RGpA"
  misc_feature 3562..4176: note = complement /label="Origin pMB1 ori (pUC)"
  misc_feature 4336..5196: note = complement /label="Bacterial Selection Amp"
  source 1..5327: mol_type = other DNA
gtcgacattgattattgactagatcatcgcgtgaggctccggtgcccgtcagtgggcagagcgcacatcgcccacagtccccgagaagttggggggaggggtcggcaattgaaccggtgcctagagaaggtggcgcggggtaaactgggaaagtgatgtcgtgtactggctccgcctttttcccgagggtgggggagaaccgtatataagtgcagtagtcgccgtgaacgttctttttcgcaacgggtttgccgccagaacacaggtaagtgccgtgtgtggttcccgcgggcctggcctctttacgggttatggcccttgcgtgccttgaattacttccacgcccctggctgcagtacgtgattcttgatcccgagcttcgggttggaagtgggtgggagagttcgaggccttgcgcttaaggagccccttcgcctcgtgcttgagttgaggcctggcctgggcgctggggccgccgcgtgcgaatctggtggcaccttcgcgcctgtctcgctgctttcgataagtctctagccatttaaaatttttgatgacctgctgcgacgctttttttctggcaagatagtcttgtaaatgcgggccaagatctgcacactggtatttcggtttttggggccgcgggcggcgacggggcccgtgcgtcccagcgcacatgttcggcgaggcggggcctgcgagcgcggccaccgagaatcggacgggggtagtctcaagctggccggcctgctctggtgcctggcctcgcgccgccgtgtatcgccccgccctgggcggcaaggctggcccggtcggcaccagttgcgtgagcggaaagatggccgcttcccggccctgctgcagggagctcaaaatggaggacgcggcgctcgggagagcgggcgggtgagtcacccacacaaaggaaaagggcctttccgtcctcagccgtcgcttcatgtgactccacggagtaccgggcgccgtccaggcacctcgattagttctcgagcttttggagtacgtcgtctttaggttggggggaggggttttatgcgatggagtttccccacactgagtgggtggagactgaagttaggccagcttggcacttgatgtaattctccttggaatttgccctttttgagtttggatcttggttcattctcaagcctcagacagtggttcaaagtttttttcttccatttcaggtgtcgtgaggaattgccaccatgaagaagcccgaactcaccgctaccagcgttgaaaaatttctcatcgagaagttcgacagtgtgagcgacctgatgcagttgtcggagggcgaagagagccgagccttcagcttcgatgtcggcggacgcggctatgtactgcgggtgaatagctgcgctgatggcttctacaaagaccgctacgtgtaccgccacttcgccagcgctgcactacccatccccgaagtgttggacatcggcgagttcagcgagagcctgacatactgcatcagtagacgcgcccaaggcgttactctccaagacctccccgaaacagagctgcctgctgtgttacagcctgtcgccgaagctatggatgctattgccgccgccgacctcagtcaaaccagcggcttcggcccattcgggccccaaggcatcggccagtacacaacctggcgggatttcatttgcgccattgctgatccccatgtctaccactggcagaccgtgatggacgacaccgtgtccgccagcgtagctcaagccctggacgaactgatgctgtgggccgaagactgtcccgaggtgcgccacctcgtccatgccgacttcggcagcaacaacgtcctgaccgacaacggccgcatcaccgccgtaatcgactggtccgaagctatgttcggggacagtcagtacgaggtggccaacatcttcttctggcggccctggctggcttgcatggagcagcagactcgctacttcgagcgccggcatcccgagctggccggcagccctcgtctgcgagcctacatgctgcgcatcggcctggatcagctctaccagagcctcgtggacggcaacttcgacgatgctgcctgggctcaaggccgctgcgatgccatcgtccgcagcggggccggcaccgtcggtcgcacacaaatcgctcgccggagcgcagccgtatggaccgacggctgcgtcgaggtgctggccgacagcggcaaccgccggcccagtacacgaccgcgcgctaaggaggtaggtcgagtttaaggccgcactcctcaggtgcaggctgcctatcagaaggtggtggctggtgtggccaatgccctggctcacaaataccactgagatctttttccctctgccaaaaattatggggacatcatgaagccccttgagcatctgacttctggctaataaaggaaatttattttcattgcaatagtgtgttggaattttttgtgtctctcactcggaaggacatatgggagggcaaatcatttaaaacatcagaatgagtatttggtttagagtttggcaacatatgccatatgctggctgccatgaacaaaggtggctataaagaggtcatcagtatatgaaacagccccctgctgtccattccttattccatagaaaagccttgacttgaggttagattttttttatattttgttttgtgttatttttttctttaacatccctaaaattttccttacatgttttactagccagatttttcctcctctcctgactactcccagtcatagctgtccctcttctcttatgaagatccctcgacctgcagcccaagcttggcgtaatcatggtcatagctgtttcctgtgtgaaattgttatccgctcacaattccacacaacatacgagccggaagcataaagtgtaaagcctggggtgcctaatgagtgagctaactcacattaattgcgttgcgctcactgcccgctttccagtcgggaaacctgtcgtgccagcggatccgcatctcaattagtcagcaaccatagtcccgcccctaactccgcccatcccgcccctaactccgcccagttccgcccattctccgccccatggctgactaattttttttatttatgcagaggccgaggccgcctcggcctctgagctattccagaagtagtgaggaggcttttttggaggcctaggcttttgcaaaaagctaacttgtttattgcagcttataatggttacaaataaagcaatagcatcacaaatttcacaaataaagcatttttttcactgcattctagttgtggtttgtccaaactcatcaatgtatcttatcatgtctggatccgctgcattaatgaatcggccaacgcgcggggagaggcggtttgcgtattgggcgctcttccgcttcctcgctcactgactcgctgcgctcggtcgttcggctgcggcgagcggtatcagctcactcaaaggcggtaatacggttatccacagaatcaggggataacgcaggaaagaacatgtgagcaaaaggccagcaaaaggccaggaaccgtaaaaaggccgcgttgctggcgtttttccataggctccgcccccctgacgagcatcacaaaaatcgacgctcaagtcagaggtggcgaaacccgacaggactataaagataccaggcgtttccccctggaagctccctcgtgcgctctcctgttccgaccctgccgcttaccggatacctgtccgcctttctcccttcgggaagcgtggcgctttctcaatgctcacgctgtaggtatctcagttcggtgtaggtcgttcgctccaagctgggctgtgtgcacgaaccccccgttcagcccgaccgctgcgccttatccggtaactatcgtcttgagtccaacccggtaagacacgacttatcgccactggcagcagccactggtaacaggattagcagagcgaggtatgtaggcggtgctacagagttcttgaagtggtggcctaactacggctacactagaaggacagtatttggtatctgcgctctgctgaagccagttaccttcggaaaaagagttggtagctcttgatccggcaaacaaaccaccgctggtagcggtggtttttttgtttgcaagcagcagattacgcgcagaaaaaaaggatctcaagaagatcctttgatcttttctacggggtctgacgctcagtggaacgaaaactcacgttaagggattttggtcatgagattatcaaaaaggatcttcacctagatccttttaaattaaaaatgaagttttaaatcaatctaaagtatatatgagtaaacttggtctgacagttaccaatgcttaatcagtgaggcacctatctcagcgatctgtctatttcgttcatccatagttgcctgactccccgtcgtgtagataactacgatacgggagggcttaccatctggccccagtgctgcaatgataccgcgagacccacgctcaccggctccagatttatcagcaataaaccagccagccggaagggccgagcgcagaagtggtcctgcaactttatccgcctccatccagtctattaattgttgccgggaagctagagtaagtagttcgccagttaatagtttgcgcaacgttgttgccattgctacaggcatcgtggtgtcacgctcgtcgtttggtatggcttcattcagctccggttcccaacgatcaaggcgagttacatgatcccccatgttgtgcaaaaaagcggttagctccttcggtcctccgatcgttgtcagaagtaagttggccgcagtgttatcactcatggttatggcagcactgcataattctcttactgtcatgccatccgtaagatgcttttctgtgactggtgagtactcaaccaagtcattctgagaatagtgtatgcggcgaccgagttgctcttgcccggcgtcaatacgggataataccgcgccacatagcagaactttaaaagtgctcatcattggaaaacgttcttcggggcgaaaactctcaaggatcttaccgctgttgagatccagttcgatgtaacccactcgtgcacccaactgatcttcagcatcttttactttcaccagcgtttctgggtgagcaaaaacaggaaggcaaaatgccgcaaaaaagggaataagggcgacacggaaatgttgaatactcatactcttcctttttcaatattattgaagcatttatcagggttattgtctcatgagcggatacatatttgaatgtatttagaaaaataaacaaataggggttccgcgcacatttccccgaaaagtgccacctg

SEQ ID NO: 2 - DNA, 927 bp, synthetic construct
  misc_feature 1..927: note = Synthetic DNA
  misc_feature 18..65: note = /label="FRT"
  misc_feature 66..342: note = complement /label="BGHpA"
  misc_feature 347..805: note = complement /label="3'Neo"
  misc_feature 806..871: note = /label="SA"
  misc_feature 872..905: note = complement /label="loxP"
  source 1..927: mol_type = other DNA
agtgccacctggtcgacgaagttcctattccgaagttcctattctctagaaagtataggaacttcccccagctggttctttccgcctcagaagccatagagcccaccgcatccccagcatgcctgctattgtcttcccaatcctcccccttgctgtcctgccccaccccaccccccagaatagaatgacacctactcagacaatgcgatgcaatttcctcattttattaggaaaggacagtgggagtggcaccttccagggtcaaggaaggcacgggggaggggcaaacaacagatggctggcaactagaaggcacagtcgaggctgatcagcgagctctaggaattcagaagaactcgtccagcagtctgtagaaggcgatccgctggctgtcaggggcggcaattccatacagcaccaggaaccggtcggcccactctccgcccagttcttcggcaatgtcccgggtggccagggcgatatcctggtatctgtcggccacgcccagtctgccgcagtcgataaagccgctgaaccggccgttttccaccatgatgttgggcaggcaggcatccccgtgtgtcacgaccagatcgtcgccgtcgggcattctggccttcagtctagcaaacagctcggcgggagccagtccctggtgttcttcatccaggtcgtcctggtccaccaggccggcttccattctggttctggcccgctcgatccggtgcttggcttgatgatcgaatggacaggtggcaggatccagggtgtgcagtctccgcatggcgtcggccatgatggacacctgtggagagaaaggcaaagtggatgtcagtaagaccaataggtgcctatcagaaacgcaagagtcataacttcgtataatgtatgctatacgaagttatgaattcgacattgattattgac

SEQ ID NO: 3 - DNA, 25 bp, synthetic construct
  misc_feature 1..25: note = Synthetic DNA
  source 1..25: mol_type = other DNA
aattagccatgtgtggtggcacacg

SEQ ID NO: 4 - DNA, 25 bp, synthetic construct
  misc_feature 1..25: note = Synthetic DNA
  source 1..25: mol_type = other DNA
ccctgagagtcctgtgcatatcagc

SEQ ID NO: 5 - DNA, 20 bp, synthetic construct
  misc_feature 1..20: note = Synthetic DNA
  source 1..20: mol_type = other DNA
tgaggcaggagaatcacttg

SEQ ID NO: 6 - DNA, 27 bp, synthetic construct
  misc_feature 1..27: note = Synthetic DNA
  source 1..27: mol_type = other DNA
gctaaggattaaatcactgcggttatc

SEQ ID NO: 7 - DNA, 39 bp, synthetic construct
  misc_feature 1..39: note = Synthetic DNA
  source 1..39: mol_type = other DNA
gacctgcagcccaagctaccagggataacaggggaacag

SEQ ID NO: 8 - DNA, 38 bp, synthetic construct
  misc_feature 1..38: note = Synthetic DNA
  source 1..38: mol_type = other DNA
gaataggaacttcgtcgactgtcaagcagctagcaggc

SEQ ID NO: 9 - DNA, 864 bp, synthetic construct
  misc_feature 1..864: note = Synthetic DNA
  misc_feature 46..111: note = /lebel="P2A" /note="P2A"
  misc_feature 118..831: note = /lebel="mRuby2"
  source 1..864: mol_type = other DNA
actactcccagtcatagctggcgcgctaaggaggtaggtcgagttggaagcggagctactaacttcagcctgctgaagcaggctggagacgtggaggagaaccctggaccttacgtaatggtgtccaagggcgaggaactgatcaaagaaaacatgcggatgaaggtcgtgatggaaggcagcgtgaacggccaccagttcaagtgtacaggcgagggcgagggcaacccctacatgggcacccagaccatgcggatcaaagtgatcgagggcggacccctgcccttcgcctttgatatcctggccaccagctttatgtacggcagcagaaccttcatcaagtaccccaagggcatccccgatttcttcaagcagagcttccccgagggcttcacctgggagagagtgaccagatacgaggacggcggcgtcgtgaccgtgatgcaggataccagcctggaagatggctgcctggtgtaccacgtgcaagtgcggggcgtgaacttccccagcaacggccctgtgatgcagaaaaagaccaagggctgggagcccaacaccgagatgatgtaccctgccgacggcggcctgagaggctacacacacatggccctgaaggtggacggcggaggccacctgagctgtagcttcgtgaccacctaccggtccaagaaaaccgtgggcaacatcaagatgcccggcatccacgccgtggaccaccggctggaaagactggaagagtccgacaacgagatgttcgtggtgcagcgcgagcatgccgtggccaagtttgctggactgggcggaggcatggacgagctgtacaaatgaggtaccgcgcgcggaggattgggaagacaatag

SEQ ID NO: 10 - DNA, 20 bp, synthetic construct
  misc_feature 1..20: note = Synthetic DNA
  source 1..20: mol_type = other DNA
actactcccagtcatagctg

SEQ ID NO: 11 - DNA, 21 bp, synthetic construct
  misc_feature 1..21: note = Synthetic DNA
  source 1..21: mol_type = other DNA
ctattgtcttcccaatcctcc

SEQ ID NO: 12 - DNA, 5009 bp, synthetic construct
  misc_feature 1..5009: note = Synthetic DNA
  misc_feature 30..1217: note = /label="EF1"
  misc_feature 1230..1949: note = /label="EGFP"
  misc_feature 1956..2490: note = /label="RGpA"
  misc_feature 3244..3858: note = complement /label="Origin pMB1 ori (pUC)"
  misc_feature 4018..4878: note = /label="Bacterial Selection Amp"
  source 1..5009: mol_type = other DNA
gtcgacattgattattgactagatcatcgcgtgaggctccggtgcccgtcagtgggcagagcgcacatcgcccacagtccccgagaagttggggggaggggtcggcaattgaaccggtgcctagagaaggtggcgcggggtaaactgggaaagtgatgtcgtgtactggctccgcctttttcccgagggtgggggagaaccgtatataagtgcagtagtcgccgtgaacgttctttttcgcaacgggtttgccgccagaacacaggtaagtgccgtgtgtggttcccgcgggcctggcctctttacgggttatggcccttgcgtgccttgaattacttccacgcccctggctgcagtacgtgattcttgatcccgagcttcgggttggaagtgggtgggagagttcgaggccttgcgcttaaggagccccttcgcctcgtgcttgagttgaggcctggcctgggcgctggggccgccgcgtgcgaatctggtggcaccttcgcgcctgtctcgctgctttcgataagtctctagccatttaaaatttttgatgacctgctgcgacgctttttttctggcaagatagtcttgtaaatgcgggccaagatctgcacactggtatttcggtttttggggccgcgggcggcgacggggcccgtgcgtcccagcgcacatgttcggcgaggcggggcctgcgagcgcggccaccgagaatcggacgggggtagtctcaagctggccggcctgctctggtgcctggcctcgcgccgccgtgtatcgccccgccctgggcggcaaggctggcccggtcggcaccagttgcgtgagcggaaagatggccgcttcccggccctgctgcagggagctcaaaatggaggacgcggcgctcgggagagcgggcgggtgagtcacccacacaaaggaaaagggcctttccgtcctcagccgtcgcttcatgtgactccacggagtaccgggcgccgtccaggcacctcgattagttctcgagcttttggagtacgtcgtctttaggttggggggaggggttttatgcgatggagtttccccacactgagtgggtggagactgaagttaggccagcttggcacttgatgtaattctccttggaatttgccctttttgagtttggatcttggttcattctcaagcctcagacagtggttcaaagtttttttcttccatttcaggtgtcgtgaggaattgccaccatggtgagcaagggcgaggagctgttcaccggggtggtgcccatcctggtcgagctggacggcgacgtaaacggccacaagttcagcgtgtccggcgagggcgagggcgatgccacctacggcaagctgaccctgaagttcatctgcaccaccggcaagctgcccgtgccctggcccaccctcgtgaccaccctgacctacggcgtgcagtgcttcagccgctaccccgaccacatgaagcagcacgacttcttcaagtccgccatgcccgaaggctacgtccaggagcgcaccatcttcttcaaggacgacggcaactacaagacccgcgccgaggtgaagttcgagggcgacaccctggtgaaccgcatcgagctgaagggcatcgacttcaaggaggacggcaacatcctggggcacaagctggagtacaactacaacagccacaacgtctatatcatggccgacaagcagaagaacggcatcaaggtgaacttcaagatccgccacaacatcgaggacggcagcgtgcagctcgccgaccactaccagcagaacacccccatcggcgacggccccgtgctgctgcccgacaaccactacctgagcacccagtccgccctgagcaaagaccccaacgagaagcgcgatcacatggtcctgctggagttcgtgaccgccgccgggatcactctcggcatggacgagctgtacaagtaaggccgcactcctcaggtgcaggctgcctatcagaaggtggtggctggtgtggccaatgccctggctcacaaataccactgagatctttttccctctgccaaaaattatggggacatcatgaagccccttgagcatctgacttctggctaataaaggaaatttattttcattgcaatagtgtgttggaattttttgtgtctctcactcggaaggacatatgggagggcaaatcatttaaaacatcagaatgagtatttggtttagagtttggcaacatatgccatatgctggctgccatgaacaaaggtggctataaagaggtcatcagtatatgaaacagccccctgctgtccattccttattccatagaaaagccttgacttgaggttagattttttttatattttgttttgtgttatttttttctttaacatccctaaaattttccttacatgttttactagccagatttttcctcctctcctgactactcccagtcatagctgtccctcttctcttatgaagatccctcgacctgcagcccaagcttggcgtaatcatggtcatagctgtttcctgtgtgaaattgttatccgctcacaattccacacaacatacgagccggaagcataaagtgtaaagcctggggtgcctaatgagtgagctaactcacattaattgcgttgcgctcactgcccgctttccagtcgggaaacctgtcgtgccagcggatccgcatctcaattagtcagcaaccatagtcccgcccctaactccgcccatcccgcccctaactccgcccagttccgcccattctccgccccatggctgactaattttttttatttatgcagaggccgaggccgcctcggcctctgagctattccagaagtagtgaggaggcttttttggaggcctaggcttttgcaaaaagctaacttgtttattgcagcttataatggttacaaataaagcaatagcatcacaaatttcacaaataaagcatttttttcactgcattctagttgtggtttgtccaaactcatcaatgtatcttatcatgtctggatccgctgcattaatgaatcggccaacgcgcggggagaggcggtttgcgtattgggcgctcttccgcttcctcgctcactgactcgctgcgctcggtcgttcggctgcggcgagcggtatcagctcactcaaaggcggtaatacggttatccacagaatcaggggataacgcaggaaagaacatgtgagcaaaaggccagcaaaaggccaggaaccgtaaaaaggccgcgttgctggcgtttttccataggctccgcccccctgacgagcatcacaaaaatcgacgctcaagtcagaggtggcgaaacccgacaggactataaagataccaggcgtttccccctggaagctccctcgtgcgctctcctgttccgaccctgccgcttaccggatacctgtccgcctttctcccttcgggaagcgtggcgctttctcaatgctcacgctgtaggtatctcagttcggtgtaggtcgttcgctccaagctgggctgtgtgcacgaaccccccgttcagcccgaccgctgcgccttatccggtaactatcgtcttgagtccaacccggtaagacacgacttatcgccactggcagcagccactggtaacaggattagcagagcgaggtatgtaggcggtgctacagagttcttgaagtggtggcctaactacggctacactagaaggacagtatttggtatctgcgctctgctgaagccagttaccttcggaaaaagagttggtagctcttgatccggcaaacaaaccaccgctggtagcggtggtttttttgtttgcaagcagcagattacgcgcagaaaaaaaggatctcaagaagatcctttgatcttttctacggggtctgacgctcagtggaacgaaaactcacgttaagggattttggtcatgagattatcaaaaaggatcttcacctagatccttttaaattaaaaatgaagttttaaatcaatctaaagtatatatgagtaaacttggtctgacagttaccaatgcttaatcagtgaggcacctatctcagcgatctgtctatttcgttcatccatagttgcctgactccccgtcgtgtagataactacgatacgggagggcttaccatctggccccagtgctgcaatgataccgcgagacccacgctcaccggctccagatttatcagcaataaaccagccagccggaagggccgagcgcagaagtggtcctgcaactttatccgcctccatccagtctattaattgttgccgggaagctagagtaagtagttcgccagttaatagtttgcgcaacgttgttgccattgctacaggcatcgtggtgtcacgctcgtcgtttggtatggcttcattcagctccggttcccaacgatcaaggcgagttacatgatcccccatgttgtgcaaaaaagcggttagctccttcggtcctccgatcgttgtcagaagtaagttggccgcagtgttatcactcatggttatggcagcactgcataattctcttactgtcatgccatccgtaagatgcttttctgtgactggtgagtactcaaccaagtcattctgagaatagtgtatgcggcgaccgagttgctcttgcccggcgtcaatacgggataataccgcgccacatagcagaactttaaaagtgctcatcattggaaaacgttcttcggggcgaaaactctcaaggatcttaccgctgttgagatccagttcgatgtaacccactcgtgcacccaactgatcttcagcatcttttactttcaccagcgtttctgggtgagcaaaaacaggaaggcaaaatgccgcaaaaaagggaataagggcgacacggaaatgttgaatactcatactcttcctttttcaatattattgaagcatttatcagggttattgtctcatgagcggatacatatttgaatgtatttagaaaaataaacaaataggggttccgcgcacatttccccgaaaagtgccacctg

SEQ ID NO: 13 - DNA, 1285 bp, synthetic construct
  misc_feature 1..1285: note = Synthetic DNA
  misc_feature 22..618: note = complement /label="Puro"
  misc_feature 619..681: note = complement /label="T2A"
  misc_feature 684..750: note = /label="SA"
  misc_feature 751..784: note = complement /label="loxP"
  misc_feature 788..854: note = /label="SD"
  misc_feature 855..1199: note = complement /label="5'Neo"
  misc_feature 1200..1265: note = complement /label="P2A"
  source 1..1285: mol_type = other DNA
tgcggccttacttgtacgaattcaggcgccaggctttctggtcatgcaccaggtggctctatccttggggcattccacgtcggcggtcacggtgaagcccagtctctcgtagaagggcaggtttctgggggcgcttgtttccaggaaggcgggcacgccagccctttcagcagcttccacgccaggcagcaccacagcagatcccagtcccttgccctggtggtcaggtgacacgcccacggtggccagaaaccaggcaggctctttaggtctgtggggggccagcaggccttccatctgctgctgggcagccagtctagagccgctcagctcggccattctaggtccgatctcggcgaacacagcgccggcttccacagactcaggggttgtccacacagccacagcggcgccatcatcggccacccacactttgccgatgtccaggcccactctggtcagaaacagttcctgcagctcggtcactctctcgatgtgtctgtcggggtccacggtgtgtctggtggcagggtaatcggcgaaggcagcggccagtgtccgcacagctctaggcacatcgtccctggtggccagccgcactgtgggcttgtactcggtaggtccaggattctcctccacgtcaccgcatgttagcagacttcctctgccctctccgcttcctacctgtggagagaaaggcaaagtggatgtcagtaagaccaataggtgcctatcagaaacgcaagagtcataacttcgtataatgtatgctatacgaagttatgaattctctgtctcgacaagcccagtttctattggtctccttaaacctgtcttgtaaccttgatacttaccttctcggcaggggccagatggctagacagcagatcctggcctggcacttcgcccagcagcagccagtctcttccggcctctgtcacgacgtccagcacagcggcacatggcacgcctgttgtggccagccagctcagtctggcggcttcatcctgcagctcgttcagggcgccagacaggtcggttttcacgaacagcacgggtctgccctgggcactcagtctgaacacggcggcatcggaacagccgatggtctgctgggcccaatcgtagccgaacagtctttccacccaggcggctggagatccggcgtgcagtccatcctgctcgatggcagagcccataggtccagggttctcctccacgtctccagcctgcttcagcaggctgaagttagtagctccgcttcccttgtacagctcgtccatgc

SEQ ID NO: 14 - DNA, 54 bp, synthetic construct
  misc_feature 1..54: note = Synthetic DNA
  source 1..54: mol_type = other DNA
tcgaggaagttcctattccgaagttcctattctctagaaagtataggaacttcg

SEQ ID NO: 15 - DNA, 54 bp, synthetic construct
  misc_feature 1..54: note = Synthetic DNA
  source 1..54: mol_type = other DNA
tcgacgaagttcctatactttctagagaataggaacttcggaataggaacttcc

SEQ ID NO: 16 - DNA, 26 bp, synthetic construct
  misc_feature 1..26: note = Synthetic DNA
  source 1..26: mol_type = other DNA
gcgtcagatctcattatggatggctg

SEQ ID NO: 17 - DNA, 26 bp, synthetic construct
  misc_feature 1..26: note = Synthetic DNA
  source 1..26: mol_type = other DNA
cgagcctatgagggtcattctcactc

SEQ ID NO: 18 - DNA, 20 bp, synthetic construct
  misc_feature 1..20: note = Synthetic DNA
  source 1..20: mol_type = other DNA
gaactcaggaccttcagaag

SEQ ID NO: 19 - DNA, 25 bp, synthetic construct
  misc_feature 1..25: note = Synthetic DNA
  source 1..25: mol_type = other DNA
caactaacacagttactcccataac

SEQ ID NO: 20 - DNA, 43 bp, synthetic construct
  misc_feature 1..43: note = Synthetic DNA
  source 1..43: mol_type = other DNA
gtataggaacttcgtcgaacgctggtaacatttgccaacatct

SEQ ID NO: 21 - DNA, 44 bp, synthetic construct
  misc_feature 1..44: note = Synthetic DNA
  source 1..44: mol_type = other DNA
acctgcagcccaagctttgttggcctgatatctcattaaatctg

SEQ ID NO: 22 - DNA, 8424 bp, synthetic construct
  misc_feature 1..8424: note = Synthetic DNA
  misc_feature 819..1679: note = /label="Amp"
  misc_feature 1839..2453: note = /label="Origin pMB1 ori (pUC)"
  misc_feature 2957..4041: note = /label="LA"
  misc_feature 4047..5746: note = /label="CAG promoter"
  misc_feature 5756..6412: note = /label="Hprt"
  misc_feature 6439..6968: note = /label="RGpA"
  misc_feature 6975..8363: note = /label="RA"
  source 1..8424: mol_type = other DNA
tatagtgagtcgtattacaattcactggccgtcgttttacaacgtcgtgactgggaaaaccctggcgttacccaacttaatcgccttgcagcacatccccctttcgccagctggcgtaatagcgaagaggcccgcaccgatcgcccttcccaacagttgcgcagcctgaatggcgaatggacgcgccctgtagcggcgcattaagcgcggcgggtgtggtggttacgcgcagcgtgaccgctacacttgccagcgccctagcgcccgctcctttcgctttcttcccttcctttctcgccacgttcgccggctttccccgtcaagctctaaatcgggggctccctttagggttccgatttagtgctttacggcacctcgaccccaaaaaacttgattagggtgatggttcacgtagtgggccatcgccctgatagacggtttttcgccctttgacgttggagtccacgttctttaatagtggactcttgttccaaactggaacaacactcaaccctatctcggtctattcttttgatttataagggattttgccgatttcggcctattggttaaaaaatgagctgatttaacaaaaatttaacgcgaattttaacaaaatattaacgcttacaatttcctgatgcggtattttctccttacgcatctgtgcggtatttcacaccgcatcaggtggcacttttcggggaaatgtgcgcggaacccctatttgtttatttttctaaatacattcaaatatgtatccgctcatgagacaataaccctgataaatgcttcaataatattgaaaaaggaagagtatgagtattcaacatttccgtgtcgcccttattcccttttttgcggcattttgccttcctgtttttgctcacccagaaacgctggtgaaagtaaaagatgctgaagatcagttgggtgcacgagtgggttacatcgaactggatctcaacagcggtaagatccttgagagttttcgccccgaagaacgttttccaatgatgagcacttttaaagttctgctatgtggcgcggtattatcccgtattgacgccgggcaagagcaactcggtcgccgcatacactattctcagaatgacttggttgagtactcaccagtcacagaaaagcatcttacggatggcatgacagtaagagaattatgcagtgctgccataaccatgagtgataacactgcggccaacttacttctgacaacgatcggaggaccgaaggagctaaccgcttttttgcacaacatgggggatcatgtaactcgccttgatcgttgggaaccggagctgaatgaagccataccaaacgacgagcgtgacaccacgatgcctgtagcaatggcaacaacgttgcgcaaactattaactggcgaactacttactctagcttcccggcaacaattaatagactggatggaggcggataaagttgcaggaccacttctgcgctcggcccttccggctggctggtttattgctgataaatctggagccggtgagcgtgggtctcgcggtatcattgcagcactggggccagatggtaagccctcccgtatcgtagttatctacacgacggggagtcaggcaactatggatgaacgaaatagacagatcgctgagataggtgcctcactgattaagcattggtaactgtcagaccaagtttactcatatatactttagattgatttaaaacttcatttttaatttaaaaggatctaggtgaagatcctttttgataatctcatgaccaaaatcccttaacgtgagttttcgttccactgagcgtcagaccccgtagaaaagatcaaaggatcttcttgagatcctttttttctgcgcgtaatctgctgcttgcaaacaaaaaaaccaccgctaccagcggtggtttgtttgccggatcaagagctaccaactctttttccgaaggtaactggcttcagcagagcgcagataccaaatactgttcttctagtgtagccgtagttaggccaccacttcaagaactctgtagcaccgcctacatacctcgctctgctaatcctgttaccagtggctgctgccagtggcgataagtcgtgtcttaccgggttggactcaagacgatagttaccggataaggcgcagcggtcgggctgaacggggggttcgtgcacacagcccagcttggagcgaacgacctacaccgaactgagatacctacagcgtgagctatgagaaagcgccacgcttcccgaagggagaaaggcggacaggtatccggtaagcggcagggtcggaacaggagagcgcacgagggagcttccagggggaaacgcctggtatctttatagtcctgtcgggtttcgccacctctgacttgagcgtcgatttttgtgatgctcgtcaggggggcggagcctatggaaaaacgccagcaacgcggcctttttacggttcctggccttttgctggccttttgctcacatgttctttcctgcgttatcccctgattctgtggataaccgtattaccgcctttgagtgagctgataccgctcgccgcagccgaacgaccgagcgcagcgagtcagtgagcgaggaagcggaagagcgcccaatacgcaaaccgcctctccccgcgcgttggccgattcattaatgcagctggcacgacaggtttcccgactggaaagcgggcagtgagcgcaacgcaattaatgtgagttagctcactcattaggcaccccaggctttacactttatgcttccggctcgtatgttgtgtggaattgtgagcggataacaatttcacacaggaaacagctatgaccatgattacgccaagctatttaggtgacactatagaatactcaagctatgcatccaacgcgttgggagctctcccatatggtcgacctgcaggcggccgcgaattcactagtgattgcctttatgtctctgggtctcatggacaaatagggttaataagagtcctgcaacaaggctgggcgtggtggctcaagcctgtaatcccagcactttgggaggtcgaggtgggcagatcacctgaggtcaggactagcctggccaacacggtgaaacctgtcaccactaaaaatacaaaattagcctggcatagtggcacatgcctgtagtcccagctactggggaggctaaggtgggagaatcacttgaactcgggaggtggaggttgcagtgagccaagatggcaccattgcactccagcctgggcgacaagagtgaaactccatctcaaaaataaataaataaataaaaataaaaatagagtcctgcaacagtgaggatgcattcagatgaaagcaacagaaaactcagctaataatgtcagttaataaagacatttaattgtttcatatttcaaaaatgtccggaggtcagcagccagtaagccccctaacgatattatctaagacccagggtctcttcatcctgctccatcatccttggcgtgctggcttttggggccctctgtgtgatactccactgatattcttggcacatgggaaacatcatctgctcttggatttcccagatcaatctgaggatattacttcttgggggtaggtagggccctgtggtggtttggactgttattcccaatcctttgcttcctccttattatttaagtgtacatccatcccctttgctgtgtgacttgcttgtgccaacagaatgtcagaggacacgatgcaagcagatgctttcaatgtgcttttgtagtttggcttggcctcttgcactcctgtgatctgacaagagaaaggcaaattccagatatccattgccccttcagctgtgacccagaatagacactggaccaggactaaaggagtcctaccaagccctgtcaagcccagcctgattagacaaaccacagacaactcacaaacccatgagcatgaaaataaatagagtggcttaagcaatctcctggggacaggtataggaggacagcaagggtccttgggttctcagagtgtcctccagctggatcctagttattaatagtaatcaattacggggtcattagttcatagcccatatatggagttccgcgttacataacttacggtaaatggcccgcctggctgaccgcccaacgacccccgcccattgacgtcaataatgacgtatgttcccatagtaacgccaatagggactttccattgacgtcaatgggtggactatttacggtaaactgcccacttggcagtacatcaagtgtatcatatgccaagtacgccccctattgacgtcaatgacggtaaatggcccgcctggcattatgcccagtacatgaccttatgggactttcctacttggcagtacatctacgtattagtcatcgctattaccatgggtcgaggtgagccccacgttctgcttcactctccccatctcccccccctccccacccccaattttgtatttatttattttttaattattttgtgcagcgatgggggcggggggggggggggcgcgcgccaggcggggcggggcggggcgaggggcggggcggggcgaggcggagaggtgcggcggcagccaatcagagcggcgcgctccgaaagtttccttttatggcgaggcggcggcggcggcggccctataaaaagcgaagcgcgcggcgggcgggagtcgctgcgttgccttcgccccgtgccccgctccgcgccgcctcgcgccgcccgccccggctctgactgaccgcgttactcccacaggtgagcgggcgggacggcccttctcctccgggctgtaattagcgcttggtttaatgacggctcgtttcttttctgtggctgcgtgaaagccttaaagggctccgggagggccctttgtgcgggggggagcggctcggggggtgcgtgcgtgtgtgtgtgcgtggggagcgccgcgtgcggcccgcgctgcccggcggctgtgagcgctgcgggcgcggcgcggggctttgtgcgctccgcgtgtgcgcgaggggagcgcggccgggggcggtgccccgcggtgcgggggggctgcgaggggaacaaaggctgcgtgcggggtgtgtgcgtgggggggtgagcagggggtgtgggcgcggcggtcgggctgtaacccccccctgcacccccctccccgagttgctgagcacggcccggcttcgggtgcggggctccgtgcggggcgtggcgcggggctcgccgtgccgggcggggggtggcggcaggtgggggtgccgggcggggcggggccgcctcgggccggggagggctcgggggaggggcgcggcggccccggagcgccggcggctgtcgaggcgcggcgagccgcagccattgccttttatggtaatcgtgcgagagggcgcagggacttcctttgtcccaaatctggcggagccgaaatctgggaggcgccgccgcaccccctctagcgggcgcgggcgaagcggtgcggcgccggcaggaaggaaatgggcggggagggccttcgtgcgtcgccgcgccgccgtccccttctccatctccagcctcggggctgccgcagggggacggctgccttcgggggggacggggcagggcggggttcggcttctggcgtgtgaccggcggctctagagcctctgctaaccatgttcatgccttcttctttttcctacagctcctgggcaacgtgctggttattgtgctgtctcatcattttggcaaagaattcaccatgccgacccgcagtcccagcgtcgtgattagcgatgatgaaccaggttatgacctagatttgttttgtatacctaatcattatgccgaggatttggaaaaagtgtttattcctcatggactgattatggacaggactgaaagacttgctcgagatgtcatgaaggagatgggaggccatcacattgtggccctctgtgtgctcaaggggggctataagttctttgctgacctgctggattacattaaagcactgaatagaaatagtgatagatccattcctatgactgtagattttatcagactgaagagctactgtaatgatcagtcaacgggggacataaaagttattggtggagatgatctctcaactttaactggaaagaatgtcttgattgttgaagatataattgacactggtaaaacaatgcaaactttgctttccctggttaagcagtacagccccaaaatggttaaggttgcaagcttgctggtgaaaaggacctctcgaagtgttggatacaggccagactttgttggatttgaaattccagacaagtttgttgttggatatgcccttgactataatgagtacttcagggatttgaatcacgtttgtgtcattagtgaaactggaaaagccaaatacaaagcctaagaattcctcgaggatatcgcggccgcactcctcaggtgcaggctgcctatcagaaggtggtggctggtgtggccaatgccctggctcacaaataccactgagatctttttccctctgccaaaaattatggggacatcatgaagccccttgagcatctgacttctggctaataaaggaaatttattttcattgcaatagtgtgttggaattttttgtgtctctcactcggaaggacatatgggagggcaaatcatttaaaacatcagaatgagtatttggtttagagtttggcaacatatgccatatgctggctgccatgaacaaaggtggctataaagaggtcatcagtatatgaaacagccccctgctgtccattccttattccatagaaaagccttgacttgaggttagattttttttatattttgttttgtgttatttttttctttaacatccctaaaattttccttacatgttttactagccagatttttcctcctctcctgactactcccagtcatagctgtccctcttctcttatgaagatccctcgaccggatccttagggcgagagaaacttcttgactcagtgacatgaattctcttaggagagtcacattagcagctctgttcagttaggagaggccagggccctgggagttcatttgttctctcctgggtgttcagcaccagatgttacttgaggggactcagttaagaaaaggctgacatagcctggcagtggtggcgcatgcctgtaatcccagcacttgggaggcagaggcaggtggatttctgagttcaaggccagcctggtctacagagtgagttccaggaccgacataaggggcaggattgagagatggctcagtggttaagagcactgactgaactttcccttccaggaggggaggggtctggtgtaattttccaaagttcatgagctgacctcttcaacatggctgttatcagggatggtttttagtgtagatatgggggaagggaggggagcgatggcagtctgaggtgagggaggggccaggatgccagggcaggggctctggataacagaacttgtgtgaatagggacagatggcgtctggaggccagcatgggctttgctgggcacccacagatacttgtttatggagagccatttgtcccttctgccagagggaagaaaaatggcttctttttgccagaggggagcaggtttcacaagttctccaggaatgctggtggttgccagaaacccttctctaggccaggttgagtgtgcctgccttttctggaagggcatgtgaggtagatcccacagggatgctatttcaggaggcagaggaaggcagatccctgtcaattcaaggccagcctggactacatgacgagttccaggccagccagggctacaggctgagaccctttctgaaaacctgtacacgaagcagcaagctgcttttttctctaagacagggtttctctgtgtagccctgactggcttggaactcagagatctgcctgcctttgcctctgcctccggcgtcctggaattaaaggcatgtgcaaccacgccagacttctcttttttttttttttttttttttgagacagggtttctctgtgtagtcctggctgtcctggaactcactgtagaccaggctggcctcaaactcagaaatccgcctgcctctgcctcccaagtgctgggattaaaggcatgcaccaccactgcctggctatgccagacttctttgtttatttgaggcaaggtctccatccggtccctcaggctgcccttgaatttggcatggagtggaggatgaccttgaactcacaactcccctgcctcccaatccccagtgttggacagaaggccgacgccacaggtggcttttgaaatgtgaaagattaaatccagggcttcctggaagacaaccacagaattcatggcaatcgaattcccgcggccgccatggcggccgggagcatgcgacgtcgggcccaattcgccc

SEQ ID NO: 23 - DNA, 554 bp, synthetic construct
  misc_feature 1..554: note = Synthetic DNA
  misc_feature 126..524: note = /label="Blasticidin resistance gene"
  source 1..554: mol_type = other DNA
cgtgtgaccggcggctctagagcctctgctaaccatgttcatgccttcttctttttcctacagctcctgggcaacgtgctggttattgtgctgtctcatcattttggcaaagtttaaacgccaccatggccaagcctttgtctcaagaagaatccaccctcattgaaagagcaacggctacaatcaacagcatccccatctctgaagactacagcgtcgccagcgcagctctctctagcgacggccgcatcttcactggtgtcaatgtatatcattttactgggggaccttgtgcagaactcgtggtgctgggcactgctgctgctgcggcagctggcaacctgacttgtatcgtcgcgatcggaaatgagaacaggggcatcttgagcccctgcggacggtgccgacaggtgcttctcgatctgcatcctgggatcaaagccatagtgaaggacagtgatggacagccgacggcagttgggattcgtgaattgctgccctctggttatgtgtgggagggctaatgtttaaacctcgaggatatcgcggccgca

SEQ ID NO: 24 - DNA, 9292 bp, synthetic construct
  misc_feature 1..9292: note = Synthetic DNA
  misc_feature 1..249: note = /label="U6 promoter"
  misc_feature 268..343: note = /label="chimeric guide RNA scaffold"
  misc_feature 344..349: note = /label="U6 terminator"
  misc_feature 440..1238: note = /label="CBh"
  misc_feature 1251..1319: note = /label="3xFLAG"
  misc_feature 1320..1370: note = /label="NLS(1)"
  misc_feature 1371..5471: note = /label="hSpCsn1"
  misc_feature 5472..5519: note = /label="NLS"
  misc_feature 5526..5588: note = /label="T2A"
  misc_feature 5589..6305: note = /label="Ametrine"
  misc_feature 6315..6546: note = /label="BGHpA"
  misc_feature 7612..8472: note = /label="Bacterial Selection Amp"
  misc_feature 8632..9246: note = /label="Origin pMB1 ori (pUC)"
  source 1..9292: mol_type = other DNA
gagggcctatttcccatgattccttcatatttgcatatacgatacaaggctgttagagagataattggaattaatttgactgtaaacacaaagatattagtacaaaatacgtgacgtagaaagtaataatttcttgggtagtttgcagttttaaaattatgttttaaaatggactatcatatgcttaccgtaacttgaaagtatttcgatttcttggctttatatatcttgtggaaaggacgaaacaccgggtcttcgagaagacctgttttagagctagaaatagcaagttaaaataaggctagtccgttatcaacttgaaaaagtggcaccgagtcggtgcttttttgttttagagctagaaatagcaagttaaaataaggctagtccgtttttagcgcgtgcgccaattctgcagacaaatggctctagaggtacccgttacataacttacggtaaatggcccgcctggctgaccgcccaacgacccccgcccattgacgtcaatagtaacgccaatagggactttccattgacgtcaatgggtggagtatttacggtaaactgcccacttggcagtacatcaagtgtatcatatgccaagtacgccccctattgacgtcaatgacggtaaatggcccgcctggcattgtgcccagtacatgaccttatgggactttcctacttggcagtacatctacgtattagtcatcgctattaccatggtcgaggtgagccccacgttctgcttcactctccccatctcccccccctccccacccccaattttgtatttatttattttttaattattttgtgcagcgatgggggcggggggggggggggggcgcgcgccaggcggggcggggcggggcgaggggcggggcggggcgaggcggagaggtgcggcggcagccaatcagagcggcgcgctccgaaagtttccttttatggcgaggcggcggcggcggcggccctataaaaagcgaagcgcgcggcgggcgggagtcgctgcgacgctgccttcgccccgtgccccgctccgccgccgcctcgcgccgcccgccccggctctgactgaccgcgttactcccacaggtgagcgggcgggacggcccttctcctccgggctgtaattagctgagcaagaggtaagggtttaagggatggttggttggtggggtattaatgtttaattacctggagcacctgcctgaaatcactttttttcaggttggaccggtgccaccatggactataaggaccacgacggagactacaaggatcatgatattgattacaaagacgatgacgataagatggccccaaagaagaagcggaaggtcggtatccacggagtcccagcagccgacaagaagtacagcatcggcctggacatcggcaccaactctgtgggctgggccgtgatcaccgacgagtacaaggtgcccagcaagaaattcaaggtgctgggcaacaccgaccggcacagcatcaagaagaacctgatcggagccctgctgttcgacagcggcgaaacagccgaggccacccggctgaagagaaccgccagaagaagatacaccagacggaagaaccggatctgctatctgcaagagatcttcagcaacgagatggccaaggtggacgacagcttcttccacagactggaagagtccttcctggtggaagaggataagaagcacgagcggcaccccatcttcggcaacatcgtggacgaggtggcctaccacgagaagtaccccaccatctaccacctgagaaagaaactggtggacagcaccgacaaggccgacctgcggctgatctatctggccctggcccacatgatcaagttccggggccacttcctgatcgagggcgacctgaaccccgacaacagcgacgtggacaagctgttcatccagctggtgcagacctacaaccagctgttcgaggaaaaccccatcaacgccagcggcgtggacgccaaggccatcctgtctgccagactgagcaagagcagacggctggaaaatctgatcgcccagctgcccggcgagaagaagaatggcctgttcggaaacctgattgccctgagcctgggcctgacccccaacttcaagagcaacttcgacctggccgaggatgccaaactgcagctgagcaaggacacctacgacgacgacctggacaacctgctggcccagatcggcgaccagtacgccgacctgtttctggccgccaagaacctgtccgacgccatcctgctgagcgacatcctgagagtgaacaccgagatcaccaaggcccccctgagcgcctctatgatcaagagatacgacgagcaccaccaggacctgaccctgctgaaagctctcgtgcggcagcagctgcctgagaagtacaaagagattttcttcgaccagagcaagaacggctacgccggctacattgacggcggagccagccaggaagagttctacaagttcatcaagcccatcctggaaaagatggacggcaccgaggaactgctcgtgaagctgaacagagaggacctgctgcggaagcagcggaccttcgacaacggcagcatcccccaccagatccacctgggagagctgcacgccattctgcggcggcaggaagatttttacccattcctgaaggacaaccgggaaaagatcgagaagatcctgaccttccgcatcccctactacgtgggccctctggccaggggaaacagcagattcgcctggatgaccagaaagagcgaggaaaccatcaccccctggaacttcgaggaagtggtggacaagggcgcttccgcccagagcttcatcgagcggatgaccaacttcgataagaacctgcccaacgagaaggtgctgcccaagcacagcctgctgtacgagtacttcaccgtgtataacgagctgaccaaagtgaaatacgtgaccgagggaatgagaaagcccgccttcctgagcggcgagcagaaaaaggccatcgtggacctgctgttcaagaccaaccggaaagtgaccgtgaagcagctgaaagaggactacttcaagaaaatcgagtgcttcgactccgtggaaatctccggcgtggaagatcggttcaacgcctccctgggcacataccacgatctgctgaaaattatcaaggacaaggacttcctggacaatgaggaaaacgaggacattctggaagatatcgtgctgaccctgacactgtttgaggacagagagatgatcgaggaacggctgaaaacctatgcccacctgttcgacgacaaagtgatgaagcagctgaagcggcggagatacaccggctggggcaggctgagccggaagctgatcaacggcatccgggacaagcagtccggcaagacaatcctggatttcctgaagtccgacggcttcgccaacagaaacttcatgcagctgatccacgacgacagcctgacctttaaagaggacatccagaaagcccaggtgtccggccagggcgatagcctgcacgagcacattgccaatctggccggcagccccgccattaagaagggcatcctgcagacagtgaaggtggtggacgagctcgtgaaagtgatgggccggcacaagcccgagaacatcgtgatcgaaatggccagagagaaccagaccacccagaagggacagaagaacagccgcgagagaatgaagcggatcgaagagggcatcaaagagctgggcagccagatcctgaaagaacaccccgtggaaaacacccagctgcagaacgagaagctgtacctgtactacctgcagaatgggcgggatatgtacgtggaccaggaactggacatcaaccggctgtccgactacgatgtggaccatatcgtgcctcagagctttctgaaggacgactccatcgacaacaaggtgctgaccagaagcgacaagaaccggggcaagagcgacaacgtgccctccgaagaggtcgtgaagaagatgaagaactactggcggcagctgctgaacgccaagctgattacccagagaaagttcgacaatctgaccaaggccgagagaggcggcctgagcgaactggataaggccggcttcatcaagagacagctggtggaaacccggcagatcacaaagcacgtggcacagatcctggactcccggatgaacactaagtacgacgagaatgacaagctgatccgggaagtgaaagtgatcaccctgaagtccaagctggtgtccgatttccggaaggatttccagttttacaaagtgcgcgagatcaacaactaccaccacgcccacgacgcctacctgaacgccgtcgtgggaaccgccctgatcaaaaagtaccctaagctggaaagcgagttcgtgtacggcgactacaaggtgtacgacgtgcggaagatgatcgccaagagcgagcaggaaatcggcaaggctaccgccaagtacttcttctacagcaacatcatgaactttttcaagaccgagattaccctggccaacggcgagatccggaagcggcctctgatcgagacaaacggcgaaaccggggagatcgtgtgggataagggccgggattttgccaccgtgcggaaagtgctgagcatgccccaagtgaatatcgtgaaaaagaccgaggtgcagacaggcggcttcagcaaagagtctatcctgcccaagaggaacagcgataagctgatcgccagaaagaaggactgggaccctaagaagtacggcggcttcgacagccccaccgtggcctattctgtgctggtggtggccaaagtggaaaagggcaagtccaagaaactgaagagtgtgaaagagctgctggggatcaccatcatggaaagaagcagcttcgagaagaatcccatcgactttctggaagccaagggctacaaagaagtgaaaaaggacctgatcatcaagctgcctaagtactccctgttcgagctggaaaacggccggaagagaatgctggcctctgccggcgaactgcagaagggaaacgaactggccctgccctccaaatatgtgaacttcctgtacctggccagccactatgagaagctgaagggctcccccgaggataatgagcagaaacagctgtttgtggaacagcacaagcactacctggacgagatcatcgagcagatcagcgagttctccaagagagtgatcctggccgacgctaatctggacaaagtgctgtccgcctacaacaagcaccgggataagcccatcagagagcaggccgagaatatcatccacctgtttaccctgaccaatctgggagcccctgccgccttcaagtactttgacaccaccatcgaccggaagaggtacaccagcaccaaagaggtgctggacgccaccctgatccaccagagcatcaccggcctgtacgagacacggatcgacctgtctcagctgggaggcgacaaaaggccggcggccacgaaaaaggccggccaggcaaaaaagaaaaaggaattcggcagtggagagggcagaggaagtctgctaacatgcggtgacgtcgaggagaatcctggcccagtgagcaagggcgaggagctgttcaccggggtggtgcccatcctggtcgagctggacggcgacgtaaacggccacaggttcagcgtgcgcggcgagggcgagggcgatgccaccaacggcaagctgaccctgaagttcatctgcacctccggcgagctgcccgtgccctggcccaccctcgtgaccaccctgtcttacggcgtgcagtgcttcgcccgctaccccgaccacatgaagcagcacgacttcttcaagtccgccatgcccgaaggctacgtccaggagcgcaccatctccttcaaggacgacggcagctacaggacccgcgccgaggtgaagttcgagggcgacaccctggtgaaccgcatcgagctgaagggcatcgacttcaaggaggacggcaacatcctggggcacaagctggagtacaacatgaacgcgtgggacgcgtatatcacggccgacaagcagaagaacggcatcaaagcgaacttcaagatcgagcacaacgtcaaggacggcggcgtgcagctcgccgacgcgtaccagcagaacacccccatcggcgacggctccgtgctgctgcctgacaaccactacctgagcttccagagcaagctgttcaaagaccccaacgagcagcgcgatcacatggtcctgctggagttcgttaccgccgccgggataactcccggcatggacgagctgtacaagtaagaattctaactagagctcgctgatcagcctcgactgtgccttctagttgccagccatctgttgtttgcccctcccccgtgccttccttgaccctggaaggtgccactcccactgtcctttcctaataaaatgaggaaattgcatcgcattgtctgagtaggtgtcattctattctggggggtggggtggggcaggacagcaagggggaggattgggaagagaatagcaggcatgctggggagcggccgcaggaacccctagtgatggagttggccactccctctctgcgcgctcgctcgctcactgaggccgggcgaccaaaggtcgcccgacgcccgggctttgcccgggcggcctcagtgagcgagcgagcgcgcagctgcctgcaggggcgcctgatgcggtattttctccttacgcatctgtgcggtatttcacaccgcatacgtcaaagcaaccatagtacgcgccctgtagcggcgcattaagcgcggcgggtgtggtggttacgcgcagcgtgaccgctacacttgccagcgccctagcgcccgctcctttcgctttcttcccttcctttctcgccacgttcgccggctttccccgtcaagctctaaatcgggggctccctttagggttccgatttagtgctttacggcacctcgaccccaaaaaacttgatttgggtgatggttcacgtagtgggccatcgccctgatagacggtttttcgccctttgacgttggagtccacgttctttaatagtggactcttgttccaaactggaacaacactcaaccctatctcgggctattcttttgatttataagggattttgccgatttcggcctattggttaaaaaatgagctgatttaacaaaaatttaacgcgaattttaacaaaatattaacgtttacaattttatggtgcactctcagtacaatctgctctgatgccgcatagttaagccagccccgacacccgccaacacccgctgacgcgccctgacgggcttgtctgctcccggcatccgcttacagacaagctgtgaccgtctccgggagctgcatgtgtcagaggttttcaccgtcatcaccgaaacgcgcgagacgaaagggcctcgtgatacgcctatttttataggttaatgtcatgataataatggtttcttagacgtcaggtggcacttttcggggaaatgtgcgcggaacccctatttgtttatttttctaaatacattcaaatatgtatccgctcatgagacaataaccctgataaatgcttcaataatattgaaaaaggaagagtatgagtattcaacatttccgtgtcgcccttattcccttttttgcggcattttgccttcctgtttttgctcacccagaaacgctggtgaaagtaaaagatgctgaagatcagttgggtgcacgagtgggttacatcgaactggatctcaacagcggtaagatccttgagagttttcgccccgaagaacgttttccaatgatgagcacttttaaagttctgctatgtggcgcggtattatcccgtattgacgccgggcaagagcaactcggtcgccgcatacactattctcagaatgacttggttgagtactcaccagtcacagaaaagcatcttacggatggcatgacagtaagagaattatgcagtgctgccataaccatgagtgataacactgcggccaacttacttctgacaacgatcggaggaccgaaggagctaaccgcttttttgcacaacatgggggatcatgtaactcgccttgatcgttgggaaccggagctgaatgaagccataccaaacgacgagcgtgacaccacgatgcctgtagcaatggcaacaacgttgcgcaaactattaactggcgaactacttactctagcttcccggcaacaattaatagactggatggaggcggataaagttgcaggaccacttctgcgctcggcccttccggctggctggtttattgctgataaatctggagccggtgagcgtggaagccgcggtatcattgcagcactggggccagatggtaagccctcccgtatcgtagttatctacacgacggggagtcaggcaactatggatgaacgaaatagacagatcgctgagataggtgcctcactgattaagcattggtaactgtcagaccaagtttactcatatatactttagattgatttaaaacttcatttttaatttaaaaggatctaggtgaagatcctttttgataatctcatgaccaaaatcccttaacgtgagttttcgttccactgagcgtcagaccccgtagaaaagatcaaaggatcttcttgagatcctttttttctgcgcgtaatctgctgcttgcaaacaaaaaaaccaccgctaccagcggtggtttgtttgccggatcaagagctaccaactctttttccgaaggtaactggcttcagcagagcgcagataccaaatactgtccttctagtgtagccgtagttaggccaccacttcaagaactctgtagcaccgcctacatacctcgctctgctaatcctgttaccagtggctgctgccagtggcgataagtcgtgtcttaccgggttggactcaagacgatagttaccggataaggcgcagcggtcgggctgaacggggggttcgtgcacacagcccagcttggagcgaacgacctacaccgaactgagatacctacagcgtgagctatgagaaagcgccacgcttcccgaagggagaaaggcggacaggtatccggtaagcggcagggtcggaacaggagagcgcacgagggagcttccagggggaaacgcctggtatctttatagtcctgtcgggtttcgccacctctgacttgagcgtcgatttttgtgatgctcgtcaggggggcggagcctatggaaaaacgccagcaacgcggcctttttacggttcctggccttttgctggccttttgctcacatgt

SEQ ID NO: 25 - DNA, 20 bp, synthetic construct
  misc_feature 1..20: note = Synthetic DNA
  source 1..20: mol_type = other DNA
ctagctgcttgacagtaacc

SEQ ID NO: 26 - DNA, 20 bp, synthetic construct
  misc_feature 1..20: note = Synthetic DNA
  source 1..20: mol_type = other DNA
gatatcaggccaacaaacgc

SEQ ID NO: 27 - DNA, 9302 bp, synthetic construct
  misc_feature 1..9302: note = Synthetic DNA
  misc_feature 1..249: note = /label="U6 promoter"
  misc_feature 268..353: note = /label="chimeric guide RNA scaffold"
  misc_feature 354..359: note = /label="U6 terminator"
  misc_feature 450..1248: note = /label="CBh"
  misc_feature 1261..1329: note = /label="3xFLAG"
  misc_feature 1330..1380: note = /label="NLS(1)"
  misc_feature 1381..5481: note = /label="hSpCsn1"
  misc_feature 5482..5529: note = /label="NLS"
  misc_feature 5536..5598: note = /label="T2A"
  misc_feature 5599..6315: note = /label="Ametrine"
  misc_feature 6325..6556: note = /label="BGHpA"
  misc_feature 7622..8482: note = /label="Bacterial Selection Amp"
  misc_feature 8642..9256: note = /label="Origine pMB1 ori (pUC)"
  source 1..9302: mol_type = other DNA
gagggcctatttcccatgattccttcatatttgcatatacgatacaaggctgttagagagataattggaattaatttgactgtaaacacaaagatattagtacaaaatacgtgacgtagaaagtaataatttcttgggtagtttgcagttttaaaattatgttttaaaatggactatcatatgcttaccgtaacttgaaagtatttcgatttcttggctttatatatcttgtggaaaggacgaaacaccgggtcttcgagaagacctgtttcagagctatgctggaaacagcatagcaagttgaaataaggctagtccgttatcaacttgaaaaagtggcaccgagtcggtgcttttttgttttagagctagaaatagcaagttaaaataaggctagtccgtttttagcgcgtgcgccaattctgcagacaaatggctctagaggtacccgttacataacttacggtaaatggcccgcctggctgaccgcccaacgacccccgcccattgacgtcaatagtaacgccaatagggactttccattgacgtcaatgggtggagtatttacggtaaactgcccacttggcagtacatcaagtgtatcatatgccaagtacgccccctattgacgtcaatgacggtaaatggcccgcctggcattgtgcccagtacatgaccttatgggactttcctacttggcagtacatctacgtattagtcatcgctattaccatggtcgaggtgagccccacgttctgcttcactctccccatctcccccccctccccacccccaattttgtatttatttattttttaattattttgtgcagcgatgggggcggggggggggggggggcgcgcgccaggcggggcggggcggggcgaggggcggggcggggcgaggcggagaggtgcggcggcagccaatcagagcggcgcgctccgaaagtttccttttatggcgaggcggcggcggcggcggccctataaaaagcgaagcgcgcggcgggcgggagtcgctgcgacgctgccttcgccccgtgccccgctccgccgccgcctcgcgccgcccgccccggctctgactgaccgcgttactcccacaggtgagcgggcgggacggcccttctcctccgggctgtaattagctgagcaagaggtaagggtttaagggatggttggttggtggggtattaatgtttaattacctggagcacctgcctgaaatcactttttttcaggttggaccggtgccaccatggactataaggaccacgacggagactacaaggatcatgatattgattacaaagacgatgacgataagatggccccaaagaagaagcggaaggtcggtatccacggagtcccagcagccgacaagaagtacagcatcggcctggacatcggcaccaactctgtgggctgggccgtgatcaccgacgagtacaaggtgcccagcaagaaattcaaggtgctgggcaacaccgaccggcacagcatcaagaagaacctgatcggagccctgctgttcgacagcggcgaaacagccgaggccacccggctgaagagaaccgccagaagaagatacaccagacggaagaaccggatctgctatctgcaagagatcttcagcaacgagatggccaaggtggacgacagcttcttccacagactggaagagtccttcctggtggaagaggataagaagcacgagcggcaccccatcttcggcaacatcgtggacgaggtggcctaccacgagaagtaccccaccatctaccacctgagaaagaaactggtggacagcaccgacaaggccgacctgcggctgatctatctggccctggcccacatgatcaagttccggggccacttcctgatcgagggcgacctgaaccccgacaacagcgacgtggacaagctgttcatccagctggtgcagacctacaaccagctgttcgaggaaaaccccatcaacgccagcggcgtggacgccaaggccatcctgtctgccagactgagcaagagcagacggctggaaaatctgatcgcccagctgcccggcgagaagaagaatggcctgttcggaaacctgattgccctgagcctgggcctgacccccaacttcaagagcaacttcgacctggccgaggatgccaaactgcagctgagcaaggacacctacgacgacgacctggacaacctgctggcccagatcggcgaccagtacgccgacctgtttctggccgccaagaacctgtccgacgccatcctgctgagcgacatcctgagagtgaacaccgagatcaccaaggcccccctgagcgcctctatgatcaagagatacgacgagcaccaccaggacctgaccctgctgaaagctctcgtgcggcagcagctgcctgagaagtacaaagagattttcttcgaccagagcaagaacggctacgccggctacattgacggcggagccagccaggaagagttctacaagttcatcaagcccatcctggaaaagatggacggcaccgaggaactgctcgtgaagctgaacagagaggacctgctgcggaagcagcggaccttcgacaacggcagcatcccccaccagatccacctgggagagctgcacgccattctgcggcggcaggaagatttttacccattcctgaaggacaaccgggaaaagatcgagaagatcctgaccttccgcatcccctactacgtgggccctctggccaggggaaacagcagattcgcctggatgaccagaaagagcgaggaaaccatcaccccctggaacttcgaggaagtggtggacaagggcgcttccgcccagagcttcatcgagcggatgaccaacttcgataagaacctgcccaacgagaaggtgctgcccaagcacagcctgctgtacgagtacttcaccgtgtataacgagctgaccaaagtgaaatacgtgaccgagggaatgagaaagcccgccttcctgagcggcgagcagaaaaaggccatcgtggacctgctgttcaagaccaaccggaaagtgaccgtgaagcagctgaaagaggactacttcaagaaaatcgagtgcttcgactccgtggaaatctccggcgtggaagatcggttcaacgcctccctgggcacataccacgatctgctgaaaattatcaaggacaaggacttcctggacaatgaggaaaacgaggacattctggaagatatcgtgctgaccctgacactgtttgaggacagagagatgatcgaggaacggctgaaaacctatgcccacctgttcgacgacaaagtgatgaagcagctgaagcggcggagatacaccggctggggcaggctgagccggaagctgatcaacggcatccgggacaagcagtccggcaagacaatcctggatttcctgaagtccgacggcttcgccaacagaaacttcatgcagctgatccacgacgacagcctgacctttaaagaggacatccagaaagcccaggtgtccggccagggcgatagcctgcacgagcacattgccaatctggccggcagccccgccattaagaagggcatcctgcagacagtgaaggtggtggacgagctcgtgaaagtgatgggccggcacaagcccgagaacatcgtgatcgaaatggccagagagaaccagaccacccagaagggacagaagaacagccgcgagagaatgaagcggatcgaagagggcatcaaagagctgggcagccagatcctgaaagaacaccccgtggaaaacacccagctgcagaacgagaagctgtacctgtactacctgcagaatgggcgggatatgtacgtggaccaggaactggacatcaaccggctgtccgactacgatgtggaccatatcgtgcctcagagctttctgaaggacgactccatcgacaacaaggtgctgaccagaagcgacaagaaccggggcaagagcgacaacgtgccctccgaagaggtcgtgaagaagatgaagaactactggcggcagctgctgaacgccaagctgattacccagagaaagttcgacaatctgaccaaggccgagagaggcggcctgagcgaactggataaggccggcttcatcaagagacagctggtggaaacccggcagatcacaaagcacgtggcacagatcctggactcccggatgaacactaagtacgacgagaatgacaagctgatccgggaagtgaaagtgatcaccctgaagtccaagctggtgtccgatttccggaaggatttccagttttacaaagtgcgcgagatcaacaactaccaccacgcccacgacgcctacctgaacgccgtcgtgggaaccgccctgatcaaaaagtaccctaagctggaaagcgagttcgtgtacggcgactacaaggtgtacgacgtgcggaagatgatcgccaagagcgagcaggaaatcggcaaggctaccgccaagtacttcttctacagcaacatcatgaactttttcaagaccgagattaccctggccaacggcgagatccggaagcggcctctgatcgagacaaacggcgaaaccggggagatcgtgtgggataagggccgggattttgccaccgtgcggaaagtgctgagcatgccccaagtgaatatcgtgaaaaagaccgaggtgcagacaggcggcttcagcaaagagtctatcctgcccaagaggaacagcgataagctgatcgccagaaagaaggactgggaccctaagaagtacggcggcttcgacagccccaccgtggcctattctgtgctggtggtggccaaagtggaaaagggcaagtccaagaaactgaagagtgtgaaagagctgctggggatcaccatcatggaaagaagcagcttcgagaagaatcccatcgactttctggaagccaagggctacaaagaagtgaaaaaggacctgatcatcaagctgcctaagtactccctgttcgagctggaaaacggccggaagagaatgctggcctctgccggcgaactgcagaagggaaacgaactggccctgccctccaaatatgtgaacttcctgtacctggccagccactatgagaagctgaagggctcccccgaggataatgagcagaaacagctgtttgtggaacagcacaagcactacctggacgagatcatcgagcagatcagcgagttctccaagagagtgatcctggccgacgctaatctggacaaagtgctgtccgcctacaacaagcaccgggataagcccatcagagagcaggccgagaatatcatccacctgtttaccctgaccaatctgggagcccctgccgccttcaagtactttgacaccaccatcgaccggaagaggtacaccagcaccaaagaggtgctggacgccaccctgatccaccagagcatcaccggcctgtacgagacacggatcgacctgtctcagctgggaggcgacaaaaggccggcggccacgaaaaaggccggccaggcaaaaaagaaaaaggaattcggcagtggagagggcagaggaagtctgctaacatgcggtgacgtcgaggagaatcctggcccagtgagcaagggcgaggagctgttcaccggggtggtgcccatcctggtcgagctggacggcgacgtaaacggccacaggttcagcgtgcgcggcgagggcgagggcgatgccaccaacggcaagctgaccctgaagttcatctgcacctccggcgagctgcccgtgccctggcccaccctcgtgaccaccctgtcttacggcgtgcagtgcttcgcccgctaccccgaccacatgaagcagcacgacttcttcaagtccgccatgcccgaaggctacgtccaggagcgcaccatctccttcaaggacgacggcagctacaggacccgcgccgaggtgaagttcgagggcgacaccctggtgaaccgcatcgagctgaagggcatcgacttcaaggaggacggcaacatcctggggcacaagctggagtacaacatgaacgcgtgggacgcgtatatcacggccgacaagcagaagaacggcatcaaagcgaacttcaagatcgagcacaacgtcaaggacggcggcgtgcagctcgccgacgcgtaccagcagaacacccccatcggcgacggctccgtgctgctgcctgacaaccactacctgagcttccagagcaagctgttcaaagaccccaacgagcagcgcgatcacatggtcctgctggagttcgttaccgccgccgggataactcccggcatggacgagctgtacaagtaagaattctaactagagctcgctgatcagcctcgactgtgccttctagttgccagccatctgttgtttgcccctcccccgtgccttccttgaccctggaaggtgccactcccactgtcctttcctaataaaatgaggaaattgcatcgcattgtctgagtaggtgtcattctattctggggggtggggtggggcaggacagcaagggggaggattgggaagagaatagcaggcatgctggggagcggccgcaggaacccctagtgatggagttggccactccctctctgcgcgctcgctcgctcactgaggccgggcgaccaaaggtcgcccgacgcccgggctttgcccgggcggcctcagtgagcgagcgagcgcgcagctgcctgcaggggcgcctgatgcggtattttctccttacgcatctgtgcggtatttcacaccgcatacgtcaaagcaaccatagtacgcgccctgtagcggcgcattaagcgcggcgggtgtggtggttacgcgcagcgtgaccgctacacttgccagcgccctagcgcccgctcctttcgctttcttcccttcctttctcgccacgttcgccggctttccccgtcaagctctaaatcgggggctccctttagggttccgatttagtgctttacggcacctcgaccccaaaaaacttgatttgggtgatggttcacgtagtgggccatcgccctgatagacggtttttcgccctttgacgttggagtccacgttctttaatagtggactcttgttccaaactggaacaacactcaaccctatctcgggctattcttttgatttataagggattttgccgatttcggcctattggttaaaaaatgagctgatttaacaaaaatttaacgcgaattttaacaaaatattaacgtttacaattttatggtgcactctcagtacaatctgctctgatgccgcatagttaagccagccccgacacccgccaacacccgctgacgcgccctgacgggcttgtctgctcccggcatccgcttacagacaagctgtgaccgtctccgggagctgcatgtgtcagaggttttcaccgtcatcaccgaaacgcgcgagacgaaagggcctcgtgatacgcctatttttataggttaatgtcatgataataatggtttcttagacgtcaggtggcacttttcggggaaatgtgcgcggaacccctatttgtttatttttctaaatacattcaaatatgtatccgctcatgagacaataaccctgataaatgcttcaataatattgaaaaaggaagagtatgagtattcaacatttccgtgtcgcccttattcccttttttgcggcattttgccttcctgtttttgctcacccagaaacgctggtgaaagtaaaagatgctgaagatcagttgggtgcacgagtgggttacatcgaactggatctcaacagcggtaagatccttgagagttttcgccccgaagaacgttttccaatgatgagcacttttaaagttctgctatgtggcgcggtattatcccgtattgacgccgggcaagagcaactcggtcgccgcatacactattctcagaatgacttggttgagtactcaccagtcacagaaaagcatcttacggatggcatgacagtaagagaattatgcagtgctgccataaccatgagtgataacactgcggccaacttacttctgacaacgatcggaggaccgaaggagctaaccgcttttttgcacaacatgggggatcatgtaactcgccttgatcgttgggaaccggagctgaatgaagccataccaaacgacgagcgtgacaccacgatgcctgtagcaatggcaacaacgttgcgcaaactattaactggcgaactacttactctagcttcccggcaacaattaatagactggatggaggcggataaagttgcaggaccacttctgcgctcggcccttccggctggctggtttattgctgataaatctggagccggtgagcgtggaagccgcggtatcattgcagcactggggccagatggtaagccctcccgtatcgtagttatctacacgacggggagtcaggcaactatggatgaacgaaatagacagatcgctgagataggtgcctcactgattaagcattggtaactgtcagaccaagtttactcatatatactttagattgatttaaaacttcatttttaatttaaaaggatctaggtgaagatcctttttgataatctcatgaccaaaatcccttaacgtgagttttcgttccactgagcgtcagaccccgtagaaaagatcaaaggatcttcttgagatcctttttttctgcgcgtaatctgctgcttgcaaacaaaaaaaccaccgctaccagcggtggtttgtttgccggatcaagagctaccaactctttttccgaaggtaactggcttcagcagagcgcagataccaaatactgtccttctagtgtagccgtagttaggccaccacttcaagaactctgtagcaccgcctacatacctcgctctgctaatcctgttaccagtggctgctgccagtggcgataagtcgtgtcttaccgggttggactcaagacgatagttaccggataaggcgcagcggtcgggctgaacggggggttcgtgcacacagcccagcttggagcgaacgacctacaccgaactgagatacctacagcgtgagctatgagaaagcgccacgcttcccgaagggagaaaggcggacaggtatccggtaagcggcagggtcggaacaggagagcgcacgagggagcttccagggggaaacgcctggtatctttatagtcctgtcgggtttcgccacctctgacttgagcgtcgatttttgtgatgctcgtcaggggggcggagcctatggaaaaacgccagcaacgcggcctttttacggttcctggccttttgctggccttttgctcacatgt

SEQ ID NO: 28 - DNA, 20 bp, synthetic construct
  misc_feature 1..20: note = Synthetic DNA
  source 1..20: mol_type = other DNA
gactcataaaccggaggagc

SEQ ID NO: 29 - DNA, 20 bp, synthetic construct
  misc_feature 1..20: note = Synthetic DNA
  source 1..20: mol_type = other DNA
cgtgtagtaggcgcccgtta

SEQ ID NO: 30 - DNA, 26 bp, synthetic construct
  misc_feature 1..26: note = Synthetic DNA
  source 1..26: mol_type = other DNA
agtaaatcctgactgagcacctcctg

SEQ ID NO: 31 - DNA, 22 bp, synthetic construct
  misc_feature 1..22: note = Synthetic DNA
  source 1..22: mol_type = other DNA
gcttgcgtgaggctgaagtgtc

SEQ ID NO: 32 - DNA, 418 bp, synthetic construct
  misc_feature 1..418: note = Synthetic DNA
  source 1..418: mol_type = other DNA
aaggagtttctgagattgcttctgtctagcttttatggaaagatatttccttttctaccataggcctcaaagcgctcttagtatacacttccaaattctacaaagagagtgttactaaaccgctctctcaaaggaaatgttaaactctatgagttgaaacacagcacacaaacagttctgagacacttctgtctgccttttatgtgaagacatccctttccaaagaatgcctccaagggttcaaaatatccacttgtagactttacaaagagagtgttcaaaactttctctaccaaaagaaaggttaaagacggtgagttcaaacgcacacatcacaaagttgtttctaagaatcatctactatgttctagagatgttcctttctatcatagctcaatgtctaaatatccactgaatc

SEQ ID NO: 33 - DNA, 27 bp, synthetic construct
  misc_feature 1..27: note = Synthetic DNA
  source 1..27: mol_type = other DNA
cttggggtccagagaagaaaatcactc

SEQ ID NO: 34 - DNA, 27 bp, synthetic construct
  misc_feature 1..27: note = Synthetic DNA
  source 1..27: mol_type = other DNA
ctctatggcttctgaggcggaaagaac

SEQ ID NO: 35 - DNA, 22 bp, synthetic construct
  misc_feature 1..22: note = Synthetic DNA
  source 1..22: mol_type = other DNA
cggagcctcacgcgatgatcta

SEQ ID NO: 36 - DNA, 29 bp, synthetic construct
  misc_feature 1..29: note = Synthetic DNA
  source 1..29: mol_type = other DNA
agtacactgtagttgtcctcagatactcc

SEQ ID NO: 37 - DNA, 26 bp, synthetic construct
  misc_feature 1..26: note = Synthetic DNA
  source 1..26: mol_type = other DNA
tccaccccaaacatttccactaactg

SEQ ID NO: 38 - DNA, 20 bp, synthetic construct
  misc_feature 1..20: note = Synthetic DNA
  source 1..20: mol_type = other DNA
tgccaggccaggatctgctg

SEQ ID NO: 39 - DNA, 20 bp, synthetic construct
  misc_feature 1..20: note = Synthetic DNA
  source 1..20: mol_type = other DNA
atccggtgcttggcttgatg

SEQ ID NO: 40 - DNA, 22 bp, synthetic construct
  misc_feature 1..22: note = Synthetic DNA
  source 1..22: mol_type = other DNA
cacatgtcccttctgccataag

SEQ ID NO: 41 - DNA, 21 bp, synthetic construct
  misc_feature 1..21: note = Synthetic DNA
  source 1..21: mol_type = other DNA
agagatcactgaagctgctac

SEQ ID NO: 42 - DNA, 22 bp, synthetic construct
  misc_feature 1..22: note = Synthetic DNA
  source 1..22: mol_type = other DNA
tctagtcccttcaagggctgag

SEQ ID NO: 43 - DNA, 24 bp, synthetic construct
  misc_feature 1..24: note = Synthetic DNA
  source 1..24: mol_type = other DNA
acaatgtctctctgaaggctgtac

SEQ ID NO: 44 - DNA, 20 bp, synthetic construct
  misc_feature 1..20: note = Synthetic DNA
  source 1..20: mol_type = other DNA
aacatcaccgtgacatgcag

SEQ ID NO: 45 - DNA, 21 bp, synthetic construct
  misc_feature 1..21: note = Synthetic DNA
  source 1..21: mol_type = other DNA
tgtctgccaatgactctgaag

SEQ ID NO: 46 - DNA, 23 bp, synthetic construct
  misc_feature 1..23: note = Synthetic DNA
  source 1..23: mol_type = other DNA
cagctgcagcaattaccggagtg

SEQ ID NO: 47 - DNA, 23 bp, synthetic construct
  misc_feature 1..23: note = Synthetic DNA
  source 1..23: mol_type = other DNA
gaagggaggcatgtcagtaggtc

SEQ ID NO: 48 - DNA, 20 bp, synthetic construct
  misc_feature 1..20: note = Synthetic DNA
  source 1..20: mol_type = other DNA
cctttgtgacagcgcacgtt

SEQ ID NO: 49 - DNA, 20 bp, synthetic construct
  misc_feature 1..20: note = Synthetic DNA
  source 1..20: mol_type = other DNA
ccagacactagggctttcgt

SEQ ID NO: 50 - DNA, 23 bp, synthetic construct
  misc_feature 1..23: note = Synthetic DNA
  source 1..23: mol_type = other DNA
cggctggatgaggtcatctccaa

SEQ ID NO: 51 - DNA, 22 bp, synthetic construct
  misc_feature 1..22: note = Synthetic DNA
  source 1..22: mol_type = other DNA
gactcaactctgggagctcatg

SEQ ID NO: 52 - DNA, 22 bp, synthetic construct
  misc_feature 1..22: note = Synthetic DNA
  source 1..22: mol_type = other DNA
gtttcaaacaggtggctcatgc